European Patent Application EP 4 434 548 A1, published September 25, 2024. Title: 双特异性抗体-喜树碱类药物偶联物及其医药用途. Applicant: 成都百利多特生物药业有限责任公司. The sequence listing filed with the application follows.

SEQUENCE LISTING (54 sequences)

SEQ ID NO: 1 - DNA, 645 bp, synthetic construct
  source 1..645: mol_type = other DNA
gacatcttgctgactcagtctccagtcatcctgtctgtgagtccaggagaaagagtcagtttctcctgcagggccagtcagagtattggcacaaacatacactggtatcagcaaagaacaaatggttctccaaggcttctcataaagtatgcttctgagtctatctctgggattccttccaggtttagtggcagtggatcagggacagattttactcttagcatcaacagtgtggagtctgaagatattgcagattattactgtcaacaaaataataactggccaaccacgttcggtgctgggaccaagctggagctgaaacgtacggtggctgcaccatctgtcttcatcttcccgccatctgatgagcagttgaaatctggaactgcctctgttgtgtgcctgctgaataacttctatcccagagaggccaaagtacagtggaaggtggataacgccctccaatcgggtaactcccaggagagtgtcacagagcaggacagcaaggacagcacctacagcctcagcagcaccctgacgctgagcaaagcagactacgagaaacacaaagtctacgcctgcgaagtcacccatcagggcctgagctcgcccgtcacaaagagcttcaacaggggagagtgttag

SEQ ID NO: 2 - protein, 214 aa, synthetic construct
DILLTQSPVILSVSPGERVSFSCRASQSIGTNIHWYQQRTNGSPRLLIKYASESISGIPSRFSGSGSGTDFTLSINSVESEDIADYYCQQNNNWPTTFGAGTKLELKRTVAAPSVFIFPPSDEQLKSGTASVVCLLNNFYPREAKVQWKVDNALQSGNSQESVTEQDSKDSTYSLSSTLTLSKADYEKHKVYACEVTHQGLSSPVTKSFNRGEC

SEQ ID NO: 3 - DNA, 2109 bp, synthetic construct
  source 1..2109: mol_type = other DNA
caggtgcagctgaagcagtcaggacctggcctagtgcagccctcacagagcctgtccatcacctgcacagtctctggtttctcattaactaactatggtgtacactgggttcgccagtctccaggaaagggtctggagtggctgggagtgatatggagtggtggaaacacagactataatacacctttcacatccagactgagcatcaacaaggacaattccaagagccaagttttctttaaaatgaacagtctgcaatctaatgacacagccatatattactgtgccagagccctcacctactatgattacgagtttgcttactggggccaagggactctggtcactgtctctagcgctagcaccaagggcccatcggtcttccccctggcaccctcctccaagagcacctctgggggcacagcggccctgggctgcctggtcaaggactacttccccgaaccggtgacggtgtcgtggaactcaggcgccctgaccagcggcgtgcacaccttcccggctgtcctacagtcctcaggactctactccctcagcagcgtggtgaccgtgccctccagcagcttgggcacccagacctacatctgcaacgtgaatcacaagcccagcaacaccaaggtggacaagagagttgagcccaaatcttgtgacaaaactcacacatgcccaccgtgcccagcacctgaactcctggggggaccgtcagtcttcctcttccccccaaaacccaaggacaccctcatgatctcccggacccctgaggtcacatgcgtggtggtggacgtgagccacgaagaccctgaggtcaagttcaactggtacgtggacggcgtggaggtgcataatgccaagacaaagccgcgggaggagcagtacaacagcacgtaccgtgtggtcagcgtcctcaccgtcctgcaccaggactggctgaatggcaaggagtacaagtgcaaggtctccaacaaagccctcccagcccccatcgagaaaaccatctccaaagccaaagggcagccccgagaaccacaggtgtacaccctgcccccatcccgggatgagctgaccaagaaccaggtcagcctgacctgcctggtcaaaggcttctatcccagcgacatcgccgtggagtgggagagcaatgggcagccggagaacaactacaagaccacgcctcccgtgctggactccgacggctccttcttcctctatagcaagctcaccgtggacaagagcaggtggcagcaggggaacgtcttctcatgctccgtgatgcatgaggctctgcacaaccactacacgcagaagagcctctccctgtctccgggtggcggtggagggtccggcggtggtggatcacaggtgcaattgcaggagtcggggggaggcctggtcaagcctggagggtccctgagactctcctgtgcagcctctggattcacctttagtagttattggatgagctgggtccgccaggctccagggaaggggctggagtgggtggccaacataaaccgcgatggaagtgcgagttactatgtggactctgtgaagggccgattcaccatctccagagacgacgccaagaactcactgtatctgcaaatgaacagcctgagagctgaggacacggctgtgtattactgtgcgagagatcgtggggtgggctacttcgatctctggggccgtggcaccctggtcaccgtctcgagcggtggaggcggttcaggcggaggtggttccggcggtggcggctcccagtctgccctgactcagcctgcctccgtgtctgggtctcctggacagtcgatcaccatctcctgcactggaaccagcagtgacgttggtggttataactttgtctcctggtaccaacaacacccaggcaaagcccccaaactcatgatctatgatgtcagtgatcggccctcaggggtgtctgatcgcttctccggctccaagtctggcaacacggcctccctgatcatctctggcctccaggctgacgacgaggctgattattactgcagctcatatgggagcagcagcactcatgtgattttcggcggagggaccaaggtgaccgtcctataa

SEQ ID NO: 4 - protein, 702 aa, synthetic construct
QVQLKQSGPGLVQPSQSLSITCTVSGFSLTNYGVHWVRQSPGKGLEWLGVIWSGGNTDYNTPFTSRLSINKDNSKSQVFFKMNSLQSNDTAIYYCARALTYYDYEFAYWGQGTLVTVSSASTKGPSVFPLAPSSKSTSGGTAALGCLVKDYFPEPVTVSWNSGALTSGVHTFPAVLQSSGLYSLSSVVTVPSSSLGTQTYICNVNHKPSNTKVDKRVEPKSCDKTHTCPPCPAPELLGGPSVFLFPPKPKDTLMISRTPEVTCVVVDVSHEDPEVKFNWYVDGVEVHNAKTKPREEQYNSTYRVVSVLTVLHQDWLNGKEYKCKVSNKALPAPIEKTISKAKGQPREPQVYTLPPSRDELTKNQVSLTCLVKGFYPSDIAVEWESNGQPENNYKTTPPVLDSDGSFFLYSKLTVDKSRWQQGNVFSCSVMHEALHNHYTQKSLSLSPGGGGGSGGGGSQVQLQESGGGLVKPGGSLRLSCAASGFTFSSYWMSWVRQAPGKGLEWVANINRDGSASYYVDSVKGRFTISRDDAKNSLYLQMNSLRAEDTAVYYCARDRGVGYFDLWGRGTLVTVSSGGGGSGGGGSGGGGSQSALTQPASVSGSPGQSITISCTGTSSDVGGYNFVSWYQQHPGKAPKLMIYDVSDRPSGVSDRFSGSKSGNTASLIISGLQADDEADYYCSSYGSSSTHVIFGGGTKVTVL

SEQ ID NO: 5 - DNA, 660 bp, synthetic construct
  source 1..660: mol_type = other DNA
gatattcaaatgactcaatctccttcttctctttctgcttctgttggtgatcgtgttactattacttgtcgttcttctcaaaatattgttcattctaatggtaatacttatcttgattggtatcaacaaactcctggtaaagctcctaaacttcttatttataaagtttctaatcgtttttctggtgttccttctcgtttttctggttctggttctggtactgattttacttttactatttcttctcttcaacctgaagatattgctacttattattgttttcaatattctcatgttccttggacttttggtcaaggtactaaacttcaaattactcgtacggtggctgcaccatctgtcttcatcttcccgccatctgatgagcagttgaaatctggaactgcctctgttgtgtgcctgctgaataacttctatcccagagaggccaaagtacagtggaaggtggataacgccctccaatcgggtaactcccaggagagtgtcacagagcaggacagcaaggacagcacctacagcctcagcagcaccctgacgctgagcaaagcagactacgagaaacacaaagtctacgcctgcgaagtcacccatcagggcctgagctcgcccgtcacaaagagcttcaacaggggagagtgttag

SEQ ID NO: 6 - protein, 219 aa, synthetic construct
DIQMTQSPSSLSASVGDRVTITCRSSQNIVHSNGNTYLDWYQQTPGKAPKLLIYKVSNRFSGVPSRFSGSGSGTDFTFTISSLQPEDIATYYCFQYSHVPWTFGQGTKLQITRTVAAPSVFIFPPSDEQLKSGTASVVCLLNNFYPREAKVQWKVDNALQSGNSQESVTEQDSKDSTYSLSSTLTLSKADYEKHKVYACEVTHQGLSSPVTKSFNRGEC

SEQ ID NO: 7 - DNA, 2121 bp, synthetic construct
  source 1..2121: mol_type = other DNA
caggtgcagctgcagcagagcggcgccgaggtgaagaagcccggcagcagcgtgaaggtgagctgcaaggccagcggctacaccttcaccaactactacatctactgggtgcggcaggcccccggccagggcctggagtggatcggcggcatcaaccccaccagcggcggcagcaacttcaacgagaagttcaagacccgggtgaccatcaccgccgacgagagcagcaccaccgcctacatggagctgagcagcctgcggagcgaggacaccgccttctacttctgcacccggcagggcctgtggttcgacagcgacggccggggcttcgacttctggggccagggcaccaccgtgaccgtgagcagcgctagcaccaagggcccatcggtcttccccctggcaccctcctccaagagcacctctgggggcacagcggccctgggctgcctggtcaaggactacttccccgaaccggtgacggtgtcgtggaactcaggcgccctgaccagcggcgtgcacaccttcccggctgtcctacagtcctcaggactctactccctcagcagcgtggtgaccgtgccctccagcagcttgggcacccagacctacatctgcaacgtgaatcacaagcccagcaacaccaaggtggacaagagagttgagcccaaatcttgtgacaaaactcacacatgcccaccgtgcccagcacctgaactcctggggggaccgtcagtcttcctcttccccccaaaacccaaggacaccctcatgatctcccggacccctgaggtcacatgcgtggtggtggacgtgagccacgaagaccctgaggtcaagttcaactggtacgtggacggcgtggaggtgcataatgccaagacaaagccgcgggaggagcagtacaacagcacgtaccgtgtggtcagcgtcctcaccgtcctgcaccaggactggctgaatggcaaggagtacaagtgcaaggtctccaacaaagccctcccagcccccatcgagaaaaccatctccaaagccaaagggcagccccgagaaccacaggtgtacaccctgcccccatcccgggatgagctgaccaagaaccaggtcagcctgacctgcctggtcaaaggcttctatcccagcgacatcgccgtggagtgggagagcaatgggcagccggagaacaactacaagaccacgcctcccgtgctggactccgacggctccttcttcctctatagcaagctcaccgtggacaagagcaggtggcagcaggggaacgtcttctcatgctccgtgatgcatgaggctctgcacaaccactacacgcagaagagcctctccctgtctccgggtggcggtggagggtccggcggtggtggatcacaggtgcaattgcaggagtcggggggaggcctggtcaagcctggagggtccctgagactctcctgtgcagcctctggattcacctttagtagttattggatgagctgggtccgccaggctccagggaaggggctggagtgggtggccaacataaaccgcgatggaagtgcgagttactatgtggactctgtgaagggccgattcaccatctccagagacgacgccaagaactcactgtatctgcaaatgaacagcctgagagctgaggacacggctgtgtattactgtgcgagagatcgtggggtgggctacttcgatctctggggccgtggcaccctggtcaccgtctcgagcggtggaggcggttcaggcggaggtggttccggcggtggcggctcccagtctgccctgactcagcctgcctccgtgtctgggtctcctggacagtcgatcaccatctcctgcactggaaccagcagtgacgttggtggttataactttgtctcctggtaccaacaacacccaggcaaagcccccaaactcatgatctatgatgtcagtgatcggccctcaggggtgtctgatcgcttctccggctccaagtctggcaacacggcctccctgatcatctctggcctccaggctgacgacgaggctgattattactgcagctcatatgggagcagcagcactcatgtgattttcggcggagggaccaaggtgaccgtcctataa

SEQ ID NO: 8 - protein, 706 aa, synthetic construct
QVQLQQSGAEVKKPGSSVKVSCKASGYTFTNYYIYWVRQAPGQGLEWIGGINPTSGGSNFNEKFKTRVTITADESSTTAYMELSSLRSEDTAFYFCTRQGLWFDSDGRGFDFWGQGTTVTVSSASTKGPSVFPLAPSSKSTSGGTAALGCLVKDYFPEPVTVSWNSGALTSGVHTFPAVLQSSGLYSLSSVVTVPSSSLGTQTYICNVNHKPSNTKVDKRVEPKSCDKTHTCPPCPAPELLGGPSVFLFPPKPKDTLMISRTPEVTCVVVDVSHEDPEVKFNWYVDGVEVHNAKTKPREEQYNSTYRVVSVLTVLHQDWLNGKEYKCKVSNKALPAPIEKTISKAKGQPREPQVYTLPPSRDELTKNQVSLTCLVKGFYPSDIAVEWESNGQPENNYKTTPPVLDSDGSFFLYSKLTVDKSRWQQGNVFSCSVMHEALHNHYTQKSLSLSPGGGGGSGGGGSQVQLQESGGGLVKPGGSLRLSCAASGFTFSSYWMSWVRQAPGKGLEWVANINRDGSASYYVDSVKGRFTISRDDAKNSLYLQMNSLRAEDTAVYYCARDRGVGYFDLWGRGTLVTVSSGGGGSGGGGSGGGGSQSALTQPASVSGSPGQSITISCTGTSSDVGGYNFVSWYQQHPGKAPKLMIYDVSDRPSGVSDRFSGSKSGNTASLIISGLQADDEADYYCSSYGSSSTHVIFGGGTKVTVL

SEQ ID NO: 9 - DNA, 1422 bp, synthetic construct
  source 1..1422: mol_type = other DNA
gacatcttgctgactcagtctccagtcatcctgtctgtgagtccaggagaaagagtcagtttctcctgcagggccagtcagagtattggcacaaacatacactggtatcagcaaagaacaaatggttctccaaggcttctcataaagtatgcttctgagtctatctctgggattccttccaggtttagtggcagtggatcagggacagattttactcttagcatcaacagtgtggagtctgaagatattgcagattattactgtcaacaaaataataactggccaaccacgttcggttgtgggaccaagctggagctgaaacgtacggtggctgcaccatctgtcttcatcttcccgccatctgatgagcagttgaaatctggaactgcctctgttgtgtgcctgctgaataacttctatcccagagaggccaaagtacagtggaaggtggataacgccctccaatcgggtaactcccaggagagtgtcacagagcaggacagcaaggacagcacctacagcctcagcagcaccctgacgctgagcaaagcagactacgagaaacacaaagtctacgcctgcgaagtcacccatcagggcctgagctcgcccgtcacaaagagcttcaacaggggagagtgtggtggcggcggaagtggcggtggaggatccggcggtggtggatcacaggtgcagctgcaggagtcggggggaggcctggtcaagcctggagggtccctgagtctctcctgtgcagcctctggattcacctttagtagttattggatgagctgggtccgccaggctccagggaaggggctggagtgggtggccaacataaaccgcgatggaagtgcgagttactatgtggactctgtgaagggccgattcaccatctccagagacgacgccaagaactcactgtatctgcaaatgaacagcctgagagctgaggacacggctgtgtattactgtgcgagagatcgtggggtgggctacttcgatctctggggccgtggcaccctggtcaccgtctcgagcggtggaggcggttcaggcggaggtggttccggcggtggcggctcccagtctgccctgactcagcctgcctccgtgtctgggtctcctggacagtcgatcaccatctcctgcactggaaccagcagtgacgttggtggttataactttgtctcctggtaccaacaacacccaggcaaagcccccaaactcatgatctatgatgtcagtgatcggccctcaggggtgtctgatcgcttctccggctccaagtctggcaacacggcctccctgatcatctctggcctccaggctgacgacgaggctgattattactgcagctcatatgggagcagcagcactcatgtgattttcggcggagggaccaaggtgaccgtcctataa

SEQ ID NO: 10 - protein, 473 aa, synthetic construct
DILLTQSPVILSVSPGERVSFSCRASQSIGTNIHWYQQRTNGSPRLLIKYASESISGIPSRFSGSGSGTDFTLSINSVESEDIADYYCQQNNNWPTTFGCGTKLELKRTVAAPSVFIFPPSDEQLKSGTASVVCLLNNFYPREAKVQWKVDNALQSGNSQESVTEQDSKDSTYSLSSTLTLSKADYEKHKVYACEVTHQGLSSPVTKSFNRGECGGGGSGGGGSGGGGSQVQLQESGGGLVKPGGSLSLSCAASGFTFSSYWMSWVRQAPGKGLEWVANINRDGSASYYVDSVKGRFTISRDDAKNSLYLQMNSLRAEDTAVYYCARDRGVGYFDLWGRGTLVTVSSGGGGSGGGGSGGGGSQSALTQPASVSGSPGQSITISCTGTSSDVGGYNFVSWYQQHPGKAPKLMIYDVSDRPSGVSDRFSGSKSGNTASLIISGLQADDEADYYCSSYGSSSTHVIFGGGTKVTVL

SEQ ID NO: 11 - DNA, 1347 bp, synthetic construct
  source 1..1347: mol_type = other DNA
caggtgcagctgaagcagtcaggacctggcctagtgcagccctcacagagcctgtccatcacctgcacagtctctggtttctcattaactaactatggtgtacactgggttcgccagtctccaggaaagtgcctggagtggctgggagtgatatggagtggtggaaacacagactataatacacctttcacatccagactgagcatcaacaaggacaattccaagagccaagttttctttaaaatgaacagtctgcaatctaatgacacagccatatattactgtgccagagccctcacctactatgattacgagtttgcttactggggccaagggactctggtcactgtctctgctgctagcaccaagggcccatcggtcttccccctggcaccctcctccaagagcacctctgggggcacagcggccctgggctgcctggtcaaggactacttccccgaaccggtgacggtgtcgtggaactcaggcgccctgaccagcggcgtgcacaccttcccggctgtcctacagtcctcaggactctactccctcagcagcgtggtgaccgtgccctccagcagcttgggcacccagacctacatctgcaacgtgaatcacaagcccagcaacaccaaggtggacaagagagttgagcccaaatcttgtgacaaaactcacacatgcccaccgtgcccagcacctgaactcctggggggaccgtcagtcttcctcttccccccaaaacccaaggacaccctcatgatctcccggacccctgaggtcacatgcgtggtggtggacgtgagccacgaagaccctgaggtcaagttcaactggtacgtggacggcgtggaggtgcataatgccaagacaaagccgcgggaggagcagtacaacagcacgtaccgtgtggtcagcgtcctcaccgtcctgcaccaggactggctgaatggcaaggagtacaagtgcaaggtctccaacaaagccctcccagcccccatcgagaaaaccatctccaaagccaaagggcagccccgagaaccacaggtgtacaccctgcccccatcccgggatgagctgaccaagaaccaggtcagcctgacctgcctggtcaaaggcttctatcccagcgacatcgccgtggagtgggagagcaatgggcagccggagaacaactacaagaccacgcctcccgtgctggactccgacggctccttcttcctctatagcaagctcaccgtggacaagagcaggtggcagcaggggaacgtcttctcatgctccgtgatgcatgaggctctgcacaaccactacacgcagaagagcctctccctgtctccgggttaa

SEQ ID NO: 12 - protein, 448 aa, synthetic construct
QVQLKQSGPGLVQPSQSLSITCTVSGFSLTNYGVHWVRQSPGKCLEWLGVIWSGGNTDYNTPFTSRLSINKDNSKSQVFFKMNSLQSNDTAIYYCARALTYYDYEFAYWGQGTLVTVSAASTKGPSVFPLAPSSKSTSGGTAALGCLVKDYFPEPVTVSWNSGALTSGVHTFPAVLQSSGLYSLSSVVTVPSSSLGTQTYICNVNHKPSNTKVDKRVEPKSCDKTHTCPPCPAPELLGGPSVFLFPPKPKDTLMISRTPEVTCVVVDVSHEDPEVKFNWYVDGVEVHNAKTKPREEQYNSTYRVVSVLTVLHQDWLNGKEYKCKVSNKALPAPIEKTISKAKGQPREPQVYTLPPSRDELTKNQVSLTCLVKGFYPSDIAVEWESNGQPENNYKTTPPVLDSDGSFFLYSKLTVDKSRWQQGNVFSCSVMHEALHNHYTQKSLSLSPG

SEQ ID NO: 13 - DNA, 645 bp, synthetic construct; identical to SEQ ID NO: 1
  source 1..645: mol_type = other DNA

SEQ ID NO: 14 - protein, 214 aa, synthetic construct; identical to SEQ ID NO: 2

SEQ ID NO: 15 - DNA, 2109 bp, synthetic construct
  source 1..2109: mol_type = other DNA
caggtgcagctgcaggagtcggggggaggcctggtcaagcctggagggtccctgagactctcctgtgcagcctctggattcacctttagtagttattggatgagctgggtccgccaggctccagggaaggggctggagtgggtggccaacataaaccgcgatggaagtgcgagttactatgtggactctgtgaagggccgattcaccatctccagagacgacgccaagaactcactgtatctgcaaatgaacagcctgagagctgaggacacggctgtgtattactgtgcgagagatcgtggggtgggctacttcgatctctggggccgtggcaccctggtcaccgtctcgagcggtggaggcggttcaggcggaggtggttccggcggtggcggctcccagtctgccctgactcagcctgcctccgtgtctgggtctcctggacagtcgatcaccatctcctgcactggaaccagcagtgacgttggtggttataactttgtctcctggtaccaacaacacccaggcaaagcccccaaactcatgatctatgatgtcagtgatcggccctcaggggtgtctgatcgcttctccggctccaagtctggcaacacggcctccctgatcatctctggcctccaggctgacgacgaggctgattattactgcagctcatatgggagcagcagcactcatgtgattttcggcggagggaccaaggtgaccgtcctaggcggtggaggatccggcggtggtggatcacaggtgcagctgaagcagtcaggacctggcctagtgcagccctcacagagcctgtccatcacctgcacagtctctggtttctcattaactaactatggtgtacactgggttcgccagtctccaggaaagggtctggagtggctgggagtgatatggagtggtggaaacacagactataatacacctttcacatccagactgagcatcaacaaggacaattccaagagccaagttttctttaaaatgaacagtctgcaatctaatgacacagccatatattactgtgccagagccctcacctactatgattacgagtttgcttactggggccaagggactctggtcactgtctctagcgctagcaccaagggcccatcggtcttccccctggcaccctcctccaagagcacctctgggggcacagcggccctgggctgcctggtcaaggactacttccccgaaccggtgacggtgtcgtggaactcaggcgccctgaccagcggcgtgcacaccttcccggctgtcctacagtcctcaggactctactccctcagcagcgtggtgaccgtgccctccagcagcttgggcacccagacctacatctgcaacgtgaatcacaagcccagcaacaccaaggtggacaagagagttgagcccaaatcttgtgacaaaactcacacatgcccaccgtgcccagcacctgaactcctggggggaccgtcagtcttcctcttccccccaaaacccaaggacaccctcatgatctcccggacccctgaggtcacatgcgtggtggtggacgtgagccacgaagaccctgaggtcaagttcaactggtacgtggacggcgtggaggtgcataatgccaagacaaagccgcgggaggagcagtacaacagcacgtaccgtgtggtcagcgtcctcaccgtcctgcaccaggactggctgaatggcaaggagtacaagtgcaaggtctccaacaaagccctcccagcccccatcgagaaaaccatctccaaagccaaagggcagccccgagaaccacaggtgtacaccctgcccccatcccgggatgagctgaccaagaaccaggtcagcctgacctgcctggtcaaaggcttctatcccagcgacatcgccgtggagtgggagagcaatgggcagccggagaacaactacaagaccacgcctcccgtgctggactccgacggctccttcttcctctatagcaagctcaccgtggacaagagcaggtggcagcaggggaacgtcttctcatgctccgtgatgcatgaggctctgcacaaccactacacgcagaagagcctctccctgtctccgggttaa

SEQ ID NO: 16 - protein, 702 aa, synthetic construct
QVQLQESGGGLVKPGGSLRLSCAASGFTFSSYWMSWVRQAPGKGLEWVANINRDGSASYYVDSVKGRFTISRDDAKNSLYLQMNSLRAEDTAVYYCARDRGVGYFDLWGRGTLVTVSSGGGGSGGGGSGGGGSQSALTQPASVSGSPGQSITISCTGTSSDVGGYNFVSWYQQHPGKAPKLMIYDVSDRPSGVSDRFSGSKSGNTASLIISGLQADDEADYYCSSYGSSSTHVIFGGGTKVTVLGGGGSGGGGSQVQLKQSGPGLVQPSQSLSITCTVSGFSLTNYGVHWVRQSPGKGLEWLGVIWSGGNTDYNTPFTSRLSINKDNSKSQVFFKMNSLQSNDTAIYYCARALTYYDYEFAYWGQGTLVTVSSASTKGPSVFPLAPSSKSTSGGTAALGCLVKDYFPEPVTVSWNSGALTSGVHTFPAVLQSSGLYSLSSVVTVPSSSLGTQTYICNVNHKPSNTKVDKRVEPKSCDKTHTCPPCPAPELLGGPSVFLFPPKPKDTLMISRTPEVTCVVVDVSHEDPEVKFNWYVDGVEVHNAKTKPREEQYNSTYRVVSVLTVLHQDWLNGKEYKCKVSNKALPAPIEKTISKAKGQPREPQVYTLPPSRDELTKNQVSLTCLVKGFYPSDIAVEWESNGQPENNYKTTPPVLDSDGSFFLYSKLTVDKSRWQQGNVFSCSVMHEALHNHYTQKSLSLSPG

SEQ ID NO: 17 - DNA, 1407 bp, synthetic construct
  source 1..1407: mol_type = other DNA
caggtgcagctgcaggagtcggggggaggcctggtcaagcctggagggtccctgagtctctcctgtgcagcctctggattcacctttagtagttattggatgagctgggtccgccaggctccagggaaggggctggagtgggtggccaacataaaccgcgatggaagtgcgagttactatgtggactctgtgaagggccgattcaccatctccagagacgacgccaagaactcactgtatctgcaaatgaacagcctgagagctgaggacacggctgtgtattactgtgcgagagatcgtggggtgggctacttcgatctctggggccgtggcaccctggtcaccgtctcgagcggtggaggcggttcaggcggaggtggttccggcggtggcggctcccagtctgccctgactcagcctgcctccgtgtctgggtctcctggacagtcgatcaccatctcctgcactggaaccagcagtgacgttggtggttataactttgtctcctggtaccaacaacacccaggcaaagcccccaaactcatgatctatgatgtcagtgatcggccctcaggggtgtctgatcgcttctccggctccaagtctggcaacacggcctccctgatcatctctggcctccaggctgacgacgaggctgattattactgcagctcatatgggagcagcagcactcatgtgattttcggcggagggaccaaggtgaccgtcctaggcggtggaggatccggcggtggtggatcagacatcttgctgactcagtctccagtcatcctgtctgtgagtccaggagaaagagtcagtttctcctgcagggccagtcagagtattggcacaaacatacactggtatcagcaaagaacaaatggttctccaaggcttctcataaagtatgcttctgagtctatctctgggattccttccaggtttagtggcagtggatcagggacagattttactcttagcatcaacagtgtggagtctgaagatattgcagattattactgtcaacaaaataataactggccaaccacgttcggttgtgggaccaagctggagctgaaacgtacggtggctgcaccatctgtcttcatcttcccgccatctgatgagcagttgaaatctggaactgcctctgttgtgtgcctgctgaataacttctatcccagagaggccaaagtacagtggaaggtggataacgccctccaatcgggtaactcccaggagagtgtcacagagcaggacagcaaggacagcacctacagcctcagcagcaccctgacgctgagcaaagcagactacgagaaacacaaagtctacgcctgcgaagtcacccatcagggcctgagctcgcccgtcacaaagagcttcaacaggggagagtgttag

SEQ ID NO: 18 - protein, 468 aa, synthetic construct
QVQLQESGGGLVKPGGSLSLSCAASGFTFSSYWMSWVRQAPGKGLEWVANINRDGSASYYVDSVKGRFTISRDDAKNSLYLQMNSLRAEDTAVYYCARDRGVGYFDLWGRGTLVTVSSGGGGSGGGGSGGGGSQSALTQPASVSGSPGQSITISCTGTSSDVGGYNFVSWYQQHPGKAPKLMIYDVSDRPSGVSDRFSGSKSGNTASLIISGLQADDEADYYCSSYGSSSTHVIFGGGTKVTVLGGGGSGGGGSDILLTQSPVILSVSPGERVSFSCRASQSIGTNIHWYQQRTNGSPRLLIKYASESISGIPSRFSGSGSGTDFTLSINSVESEDIADYYCQQNNNWPTTFGCGTKLELKRTVAAPSVFIFPPSDEQLKSGTASVVCLLNNFYPREAKVQWKVDNALQSGNSQESVTEQDSKDSTYSLSSTLTLSKADYEKHKVYACEVTHQGLSSPVTKSFNRGEC

SEQ ID NO: 19 - DNA, 1347 bp, synthetic construct; identical to SEQ ID NO: 11
  source 1..1347: mol_type = other DNA

SEQ ID NO: 20 - protein, 448 aa, synthetic construct; identical to SEQ ID NO: 12

SEQ ID NO: 21 - DNA, 1437 bp, synthetic construct
  source 1..1437: mol_type = other DNA
gatattcaaatgactcaatctccttcttctctttctgcttctgttggtgatcgtgttactattacttgtcgttcttctcaaaatattgttcattctaatggtaatacttatcttgattggtatcaacaaactcctggtaaagctcctaaacttcttatttataaagtttctaatcgtttttctggtgttccttctcgtttttctggttctggttctggtactgattttacttttactatttcttctcttcaacctgaagatattgctacttattattgttttcaatattctcatgttccttggacttttggttgcggtactaaacttcaaattactcgtacggtggctgcaccatctgtcttcatcttcccgccatctgatgagcagttgaaatctggaactgcctctgttgtgtgcctgctgaataacttctatcccagagaggccaaagtacagtggaaggtggataacgccctccaatcgggtaactcccaggagagtgtcacagagcaggacagcaaggacagcacctacagcctcagcagcaccctgacgctgagcaaagcagactacgagaaacacaaagtctacgcctgcgaagtcacccatcagggcctgagctcgcccgtcacaaagagcttcaacaggggagagtgtggtggcggcggaagtggcggtggaggatccggcggtggtggatcacaggtgcagctgcaggagtcggggggaggcctggtcaagcctggagggtccctgagtctctcctgtgcagcctctggattcacctttagtagttattggatgagctgggtccgccaggctccagggaaggggctggagtgggtggccaacataaaccgcgatggaagtgcgagttactatgtggactctgtgaagggccgattcaccatctccagagacgacgccaagaactcactgtatctgcaaatgaacagcctgagagctgaggacacggctgtgtattactgtgcgagagatcgtggggtgggctacttcgatctctggggccgtggcaccctggtcaccgtctcgagcggtggaggcggttcaggcggaggtggttccggcggtggcggctcccagtctgccctgactcagcctgcctccgtgtctgggtctcctggacagtcgatcaccatctcctgcactggaaccagcagtgacgttggtggttataactttgtctcctggtaccaacaacacccaggcaaagcccccaaactcatgatctatgatgtcagtgatcggccctcaggggtgtctgatcgcttctccggctccaagtctggcaacacggcctccctgatcatctctggcctccaggctgacgacgaggctgattattactgcagctcatatgggagcagcagcactcatgtgattttcggcggagggaccaaggtgaccgtcctataa

SEQ ID NO: 22 - protein, 478 aa, synthetic construct
DIQMTQSPSSLSASVGDRVTITCRSSQNIVHSNGNTYLDWYQQTPGKAPKLLIYKVSNRFSGVPSRFSGSGSGTDFTFTISSLQPEDIATYYCFQYSHVPWTFGCGTKLQITRTVAAPSVFIFPPSDEQLKSGTASVVCLLNNFYPREAKVQWKVDNALQSGNSQESVTEQDSKDSTYSLSSTLTLSKADYEKHKVYACEVTHQGLSSPVTKSFNRGECGGGGSGGGGSGGGGSQVQLQESGGGLVKPGGSLSLSCAASGFTFSSYWMSWVRQAPGKGLEWVANINRDGSASYYVDSVKGRFTISRDDAKNSLYLQMNSLRAEDTAVYYCARDRGVGYFDLWGRGTLVTVSSGGGGSGGGGSGGGGSQSALTQPASVSGSPGQSITISCTGTSSDVGGYNFVSWYQQHPGKAPKLMIYDVSDRPSGVSDRFSGSKSGNTASLIISGLQADDEADYYCSSYGSSSTHVIFGGGTKVTVL

SEQ ID NO: 23 - DNA, 1359 bp, synthetic construct
  source 1..1359: mol_type = other DNA
caggtgcagctgcagcagagcggcgccgaggtgaagaagcccggcagcagcgtgaaggtgagctgcaaggccagcggctacaccttcaccaactactacatctactgggtgcggcaggcccccggccagtgtctggagtggatcggcggcatcaaccccaccagcggcggcagcaacttcaacgagaagttcaagacccgggtgaccatcaccgccgacgagagcagcaccaccgcctacatggagctgagcagcctgcggagcgaggacaccgccttctacttctgcacccggcagggcctgtggttcgacagcgacggccggggcttcgacttctggggccagggcaccaccgtgaccgtgagcagcgctagcaccaagggcccatcggtcttccccctggcaccctcctccaagagcacctctgggggcacagcggccctgggctgcctggtcaaggactacttccccgaaccggtgacggtgtcgtggaactcaggcgccctgaccagcggcgtgcacaccttcccggctgtcctacagtcctcaggactctactccctcagcagcgtggtgaccgtgccctccagcagcttgggcacccagacctacatctgcaacgtgaatcacaagcccagcaacaccaaggtggacaagagagttgagcccaaatcttgtgacaaaactcacacatgcccaccgtgcccagcacctgaactcctggggggaccgtcagtcttcctcttccccccaaaacccaaggacaccctcatgatctcccggacccctgaggtcacatgcgtggtggtggacgtgagccacgaagaccctgaggtcaagttcaactggtacgtggacggcgtggaggtgcataatgccaagacaaagccgcgggaggagcagtacaacagcacgtaccgtgtggtcagcgtcctcaccgtcctgcaccaggactggctgaatggcaaggagtacaagtgcaaggtctccaacaaagccctcccagcccccatcgagaaaaccatctccaaagccaaagggcagccccgagaaccacaggtgtacaccctgcccccatcccgggatgagctgaccaagaaccaggtcagcctgacctgcctggtcaaaggcttctatcccagcgacatcgccgtggagtgggagagcaatgggcagccggagaacaactacaagaccacgcctcccgtgctggactccgacggctccttcttcctctatagcaagctcaccgtggacaagagcaggtggcagcaggggaacgtcttctcatgctccgtgatgcatgaggctctgcacaaccactacacgcagaagagcctctccctgtctccgggttaa

SEQ ID NO: 24 - protein, 452 aa, synthetic construct
QVQLQQSGAEVKKPGSSVKVSCKASGYTFTNYYIYWVRQAPGQCLEWIGGINPTSGGSNFNEKFKTRVTITADESSTTAYMELSSLRSEDTAFYFCTRQGLWFDSDGRGFDFWGQGTTVTVSSASTKGPSVFPLAPSSKSTSGGTAALGCLVKDYFPEPVTVSWNSGALTSGVHTFPAVLQSSGLYSLSSVVTVPSSSLGTQTYICNVNHKPSNTKVDKRVEPKSCDKTHTCPPCPAPELLGGPSVFLFPPKPKDTLMISRTPEVTCVVVDVSHEDPEVKFNWYVDGVEVHNAKTKPREEQYNSTYRVVSVLTVLHQDWLNGKEYKCKVSNKALPAPIEKTISKAKGQPREPQVYTLPPSRDELTKNQVSLTCLVKGFYPSDIAVEWESNGQPENNYKTTPPVLDSDGSFFLYSKLTVDKSRWQQGNVFSCSVMHEALHNHYTQKSLSLSPG

SEQ ID NO: 25 - protein, 11 aa, synthetic construct
RASQSIGTNIH

SEQ ID NO: 26 - protein, 7 aa, synthetic construct
YASESIS

SEQ ID NO: 27 - protein, 9 aa, synthetic construct
QQNNNWPTT

SEQ ID NO: 28 - protein, 107 aa, synthetic construct
DILLTQSPVILSVSPGERVSFSCRASQSIGTNIHWYQQRTNGSPRLLIKYASESISGIPSRFSGSGSGTDFTLSINSVESEDIADYYCQQNNNWPTTFGAGTKLELK

SEQ ID NO: 29 - protein, 5 aa, synthetic construct
NYGVH

SEQ ID NO: 30 - protein, 16 aa, synthetic construct
VIWSGGNTDYNTPFTS

SEQ ID NO: 31 - protein, 11 aa, synthetic construct
ALTYYDYEFAY

SEQ ID NO: 32 - protein, 5 aa, synthetic construct
SYWMS

SEQ ID NO: 33 - protein, 17 aa, synthetic construct
NINRDGSASYYVDSVKG

SEQ ID NO: 34 - protein, 9 aa, synthetic construct
DRGVGYFDL

SEQ ID NO: 35 - protein, 14 aa, synthetic construct
TGTSSDVGGYNFVS

SEQ ID NO: 36 - protein, 7 aa, synthetic construct
DVSDRPS

SEQ ID NO: 37 - protein, 11 aa, synthetic construct
SSYGSSSTHVI

SEQ ID NO: 38 - protein, 119 aa, synthetic construct
QVQLKQSGPGLVQPSQSLSITCTVSGFSLTNYGVHWVRQSPGKGLEWLGVIWSGGNTDYNTPFTSRLSINKDNSKSQVFFKMNSLQSNDTAIYYCARALTYYDYEFAYWGQGTLVTVSS

SEQ ID NO: 39 - protein, 118 aa, synthetic construct
QVQLQESGGGLVKPGGSLRLSCAASGFTFSSYWMSWVRQAPGKGLEWVANINRDGSASYYVDSVKGRFTISRDDAKNSLYLQMNSLRAEDTAVYYCARDRGVGYFDLWGRGTLVTVSS

SEQ ID NO: 40 - protein, 111 aa, synthetic construct
QSALTQPASVSGSPGQSITISCTGTSSDVGGYNFVSWYQQHPGKAPKLMIYDVSDRPSGVSDRFSGSKSGNTASLIISGLQADDEADYYCSSYGSSSTHVIFGGGTKVTVL

SEQ ID NO: 41 - protein, 16 aa, synthetic construct
RSSQNIVHSNGNTYLD

SEQ ID NO: 42 - protein, 7 aa, synthetic construct
KVSNRFS

SEQ ID NO: 43 - protein, 9 aa, synthetic construct
FQYSHVPWT

SEQ ID NO: 44 - protein, 112 aa, synthetic construct [sequence omitted]

SEQ ID NO: 45 - protein, 5 aa, synthetic construct
NYYIY

SEQ ID NO: 46 - protein, 17 aa, synthetic construct
GINPTSGGSNFNEKFKT

SEQ ID NO: 47 - protein, 14 aa, synthetic construct
QGLWFDSDGRGFDF

SEQ ID NO: 48 - protein, 123 aa, synthetic construct [sequence omitted]

SEQ ID NO: 49 - protein, 107 aa, synthetic construct
DILLTQSPVILSVSPGERVSFSCRASQSIGTNIHWYQQRTNGSPRLLIKYASESISGIPSRFSGSGSGTDFTLSINSVESEDIADYYCQQNNNWPTTFGCGTKLELK

SEQ ID NO: 50 - protein, 118 aa, synthetic construct
QVQLQESGGGLVKPGGSLSLSCAASGFTFSSYWMSWVRQAPGKGLEWVANINRDGSASYYVDSVKGRFTISRDDAKNSLYLQMNSLRAEDTAVYYCARDRGVGYFDLWGRGTLVTVSS

SEQ ID NO: 51 - protein, 111 aa, synthetic construct; identical to SEQ ID NO: 40

SEQ ID NO: 52 - protein, 119 aa, synthetic construct
QVQLKQSGPGLVQPSQSLSITCTVSGFSLTNYGVHWVRQSPGKCLEWLGVIWSGGNTDYNTPFTSRLSINKDNSKSQVFFKMNSLQSNDTAIYYCARALTYYDYEFAYWGQGTLVTVSA

SEQ ID NO: 53 - protein, 112 aa, synthetic construct
DIQMTQSPSSLSASVGDRVTITCRSSQNIVHSNGNTYLDWYQQTPGKAPKLLIYKVSNRFSGVPSRFSGSGSGTDFTFTISSLQPEDIATYYCFQYSHVPWTFGCGTKLQIT

SEQ ID NO: 54 - protein, 123 aa, synthetic construct
QVQLQQSGAEVKKPGSSVKVSCKASGYTFTNYYIYWVRQAPGQCLEWIGGINPTSGGSNFNEKFKTRVTITADESSTTAYMELSSLRSEDTAFYFCTRQGLWFDSDGRGFDFWGQGTTVTVSS